European Patent Specification EP 4 182 446 B1, published April 2, 2025. Title: Method of purifying whole virus particles. Applicant: Københavns Universitet Hvidovre Hospital Technische Hochschule Mittelhessen, Institute für Bioverfahrenstechnik und Pharmazeutische Technologie (IBPT). The sequence listing filed with the application follows.

SEQUENCE LISTING (7 sequences)

SEQ ID NO: 1 - protein, 3011 aa, Hepatitis C virus
MSTNPKPQRKTKRNTNRRPQDVKFPGGGQIVGGVYLLPRRGPRLGVRATRKTSERSQPRGRRQPIPKARRPEGRTWAQPGYPWPLYGNEGCGWAGWLLSPRGSRPSWGPTDPRRRSRNLGKVIDTLTCGFADLMGYIPLVGAPLGGAARALAHGVRVLEDGVNYATGNLPGCSFSIFLLALLSCLTGPASAYQVRNSTGLYHVTNDCPNSSIVFEAADAILHTPGCVPCVREGNASRCWVAVTPTVATRDGKLPTTQLRRHIDLLVGSATLCSALYVGDLCGSVFLVGQLFTFSPRRHWTTQDCNCSIYPGHISGHRMAWDMMMNWSPTAALLVAQLLRIPQAILDMIAGAHWGVLAGMAYFSMVGNWAKVLVVLLLFAGVDAETYVTGGSAARTTAGLASLFSPGAKQNIQLVNTNGSWHINSTALNCNDSLNTGWIAGLFYHHKFNSSGCSERLASCRPLTDFAQGWGPISHADGSGPDQRPYCWHYPPKPCGIVPAKSVCGPVYCFTPSPVVVGTTDRSGAPTYSWGANDTDVFVLNNTRPPLGNWFGCTWMNSTGFTKVCGAPPCVIGGVGNNTLRCPTDCFRKHPEATYSRCGSGPWITPRCLVDYPYRLWHYPCTINYTVFKVRMYVGGVEHRLEAACNWTRGDRCNLDDRDRSELSPLLLSTTQWQVLPCSFTTLPALSTGLIHLHQNIVDVQYLYGVGSSIASWAIKWEYVVLLFLLLADARVCSCLWMMLLISQVEAALENLVVLNAASLAGTHGLVSFLVFFCFAWYLKGKWVPGAVYALYGMWPLLLLLLALPQRAYALDTEVAASCGGVVLVGLMALTLSPYYKRYISWCLWWLQYFLTRIEAQLHVWIPPLNVRGGRDAVILLMCVVHPALVFDITKLLLAAFGPLWILQASLLKVPYFVRVQGLLRICALARKMAGGHYVQMAIIKLGALTGTYVYNHLTPLRDWAHNGLRDLAVAVEPVVFSRMETKLITWGADTAACGDIINGLPVSARRGREILLGPADGMVSKGWRLLAPITAYAQQTRGLLGCIITSLTGRDKNQVEGEIQIVSTAAQTFLATCINGVCWTVYHGAGTRTIASPKGPVIQMYTNVDKDLVGWPAPQGARSLTPCTCGSSDLYLVTRHADVIPVRRRGDSRGSLLSPRPISYLKGSSGGPLLCPAGHAVGLFRAAVCTRGVAKAVDFIPVENLETTMRSPVFTDNSSPPAVPQSFQVGHLHAPTGSGKSTKVPAAYAAQGYKVLVLNPSVAATLGFGAYMSKAHGVDPNIRTGVRTITTGSPITYSTYGKFLADGGCSGGAYDIIICDECHSTDATSILGIGTVLDQAETAGARLVVLATATPPGSITVPHPNIEEVALSTTGEIPFYGKAIPLEAIKGGRHLIFCHSKKKCDELAAKLVALGINAVAYYRGLDVSVIPTSGDVVVVATDALMTGYTGDFDSVIDCNTCVTQTVDLSLDPTFTIETTTLPQDAVSRTQRRGRTGRGKPGIYRFVALGERPSGMFDSSVLCECYDAGCAWYELTPAETTVRLRAYMNTPGLPVCQDHLEFWEGVFTGLTHIDAHFLSQTKQSGENFPYLVAYQATVCARAQAPPPSWDQMWKCLTRLKPTLHGPTPLLYRLGAVQNEVTLTHPITKYIMTCMSADLEVVTSTWVLVGGVLAALASYCLSTGCVVIVGRIVLSGKPAIIPDREVLYREFDEMEECSQHLPYIEQGMMLAEQFKQKALGLLQTASRQAEVVAPAVQTNWQKLEAFWAKHMWNFISGIHYLAGLSTLPGNPAIASLMAFTAAVTSPLTTSQTLLFNILGGWVAAQLAAPGAATAFVGAGLAGAAIGSVGLGKVLVDILAGYGAGVAGALVAFKIMSGEVPSTEDLVNLLPAILSPGALVVGVVCAAILRRHVGPGEGAVQWMNRLIAFASRGTHVSPTHYVPESDAAARVTTILSSLTVTQLLRRLHQWISSECTTPCSGSWLRDIWDWICEVLSDFKTWLKAKLMPQLPGIPFVSCQRGYKGVWRGDGIMHTRCHCGAEITGHVKNGTMRIVGPKTCRNMWSGTFPINAYTTGPCTPLPAPNYTFALWRVSAEEYVEIRQVGDFHYVTGMTTDNLKCPCQVPSPEFFTELDGVRLHRFAPPCKPLLREEVSFRVGLHEYPVGSQLPCEPEPDVAVLTSMLTDPSHITAEAAGRRLARGSPPSMASSSASQLSAPSLRATCTTNHDSPDAELIEANLLWRQEMGGNITRVESENKVVILDSFDPLVAEEDEREVSVPAEILRKSRKFTPALPIWARPDYNPPLVEPWKKPDYEPPVVHGCPLPPPQSPPVPPPRKKRTVILTESTLPTALAELATKSFGSSSTSGITGDDTTTSPEPASSSCPPDSDAESYSSMPPLEGEPGDPDLSDGSWSTVSSEADKEDVVCCSMSYTWTGALVTPCAAEEQKLPINALSNSLLRHHNLVYSTTSRSACQRQKKVTFDRLQVLDSHYQDVLKEVKAAASKVKANLLSVEEACSLTPPHSAKSKFGYGAKDVRCHARKAVNHINSVWKDLLEDSVTPIDTTIMAKNEVFCVQPEKGGRKPARLIVFPDLGVRVCEKMALYDVVSKLPLAVMGSSYGFQYSPGQRVEFLVQAWKSKKTPMGFSYDTRCFDSTVTENDIRTEEAIYQCCDLDPQARVAIKSLTERLYVGGPLTNSRGENCGYRRCRASGVLTTSCGNTLTCYIKARAACRAAGLQDCTMLVCGDDLVVICESAGVQEDAASLRAFTEAMTRYSAPPGDPPQPEYDLELITSCSSNVSVAHDGAGKRVYYLTRDPTTPLARAAWETARHTPVNSWLGNIIMFAPTLWARMILMTHFFSVLIARDQLEQALDCEIYGACYSIEPLDLPPIIQRLHGLSAFSLHSYSPGEINRVAACLRKLGVPPLRAWRHRARNVRARLLSRGGRAAICGKYLFNWAVRTKLKLTPIAAAGRLDLSGWFTAGYSGGGIFHSVSHARPRWFWSCLLLLAAGVGIYLLPNR

SEQ ID NO: 2 - DNA, 9599 bp, Hepatitis C virus
gccagccccctgatgggggcgacactccaccatgaatcactcccctgtgaggaactactgtcttcacgcagaaagcgtctagccatggcgttagtatgagtgtcgtgcagcctccaggaccccccctcccgggagagccatagtggtctgcggaaccggtgagtacaccggaattgccaggacgaccgggtcctttcttggatcaacccgctcaatgcctggagatttgggcgtgcccccgcaagactgctagccgagtagtgttgggtcgcgaaaggccttgtggtactgcctgatagggtgcttgcgagtgccccgggaggtctcgtagaccgtgcaccatgagcacgaatcctaaacctcaaagaaaaaccaaacgtaacaccaaccgtcgcccacaggacgtcaagttcccgggtggcggtcagatcgttggtggagtttacttgttgccgcgcaggggccctagattgggtgtgcgcgcgacgaggaagacttccgagcggtcgcaacctcgaggtagacgtcagcctatccccaaggcgcgtcggcccgagggcaggacctgggctcagcccgggtacccttggcccctctatggcaatgagggttgcgggtgggcgggatggctcctgtctccccgtggctctcggcctagctggggccccacggacccccggcgtaggtcgcgcaatttgggtaaggtcatcgatacccttacgtgcggcttcgccgacctcatggggtacataccgctcgtcggcgcccctcttggaggcgctgccagggccctggcgcatggcgtccgggttttggaagacggcgtgaactatgcaacagggaaccttcctggttgctctttctctattttccttctggccctgctctcttgtctgactggacccgcttcagcctaccaagtgcgcaactccacggggctttaccatgtcaccaatgattgccccaactcgagcattgtgttcgaggcggctgatgccatcctgcacactccggggtgtgtcccttgcgtacgcgagggtaacgcctcgaggtgttgggtggcggtaacccccacggtggccaccagggatggcaaactccccacaacgcagcttcgacgtcacatcgatctgcttgtcgggagcgccaccctctgctcggccctttacgtgggggacctgtgcgggtctgtctttcttgttggtcaactgttcaccttctctcccaggcgccactggacgacgcaagattgcaattgttctatctaccccggccatatttcaggtcaccgtatggcatgggatatgatgatgaactggtcccctacggcggcgttgttggtagctcagctgctccggatcccacaagccatcctggacatgatcgctggtgctcactggggagtcctggcgggcatggcgtatttctccatggtggggaactgggcgaaggttctggtagtgctgctgctatttgccggcgtcgacgcggaaacctacgtcaccgggggaagtgccgcccgtactacggctggacttgctagtcttttctcaccaggcgccaagcagaacatccagctggtcaacaccaacggcagttggcacatcaatagcacggccttgaactgcaatgacagcctcaacaccggctggatagcaggacttttctatcaccacaaattcaactcttcgggctgttccgagaggttagccagctgccgaccccttaccgattttgcccagggctggggccctatcagtcacgccgacggaagtggccccgaccaacgcccctactgctggcactaccctccaaaaccttgtggtattgtgcccgcaaagagcgtgtgtggcccggtatattgtttcactcccagtcccgtggtggtgggaacgaccgacaggtcgggcgcgcctacctacagctggggtgcaaatgacacggacgtcttcgtccttaacaacaccaggccaccgctgggcaattggttcggttgcacctggatgaactcaactggattcaccaaagtgtgcggagcgcccccttgcgtcatcggaggggtgggcaacaacaccttgcgctgccccactgattgtttccgcaagcatccggaagccacatactctcggtgcggctccggtccctggattacgcccaggtgcctggtcgactacccgtataggctttggcattatccttgtaccatcaactacaccgtgtttaaagtcaggatgtacgtgggaggggtcgagcacaggctggaagctgcctgcaactggacgcggggcgaccgttgtaatctggatgacagggacaggtccgagctcagcccgctgctgctgtccactacgcagtggcaggtcctcccgtgttccttcacgaccctgccagccttgtccaccggcctcatccacctccaccaaaacatcgtggacgtgcaatacttgtacggggtgggatcaagcatcgcgtcctgggccatcaagtgggaatacgtcgttctcttgttccttctgcttgcagacgcgcgcgtctgctcctgcttgtggatgatgttactcatatcccaagtggaggcggctttggagaacctcgtagtactcaatgcagcatccctggccgggacacacggtcttgtatccttcctcgtgttcttctgctttgcatggtatctgaagggtaagtgggtgcccggagcggtctacgccctctacgggatgtggcctctcctcttgctcctgttagcgttgccccagcgggcatacgcactggacacggaggtggccgcgtcgtgtggcggcgttgttcttgtcgggttaatggcgctgactctgtcaccatattacaagcgctatatcagctggtgcttgtggtggcttcagtatttcctgaccagaatagaagcgcaactgcacgtgtggattccccctctcaacgtccggggggggcgcgatgccgtcatcttactcatgtgtgttgtgcacccggctctggtatttgacatcaccaagctactgctggctgccttcgggcccctttggattcttcaagccagtttgcttaaggtaccctacttcgtgcgcgttcaaggccttctccggatctgcgcgctagcgcggaagatggctggaggccattacgtgcaaatggccatcatcaagttaggggcgcttactggcacttatgtttacaaccatctcaccccccttcgggactgggcgcacaacggcctgcgagatctggccgtggctgtggagccagtcgtcttctcccgaatggagaccaagcttatcacctggggggcagacaccgccgcgtgcggtgacatcatcaacggcttgcccgtctccgcccggaggggccgggagatactgctcgggccagccgatggaatggtctccaaggggtggagattgctggcgcccatcacggcgtacgcccagcaaacgaggggcctcctagggtgtataatcaccagtctgaccggccgggacaaaaaccaagtggagggtgagatccagattgtgtcaactgctgcccaaaccttcctggcaacgtgcatcaacggggtttgctggaccgtctaccacggggccggaacgaggaccatcgcatcacccaagggtccggttatccaaatgtataccaatgtggacaaagaccttgtgggctggcccgctcctcaaggtgcccgctcactgacaccctgtacctgcggctcctcggacctttacctggtcacgaggcacgccgatgtcattcccgtgcgccggcggggtgatagcaggggcagcctgctttcgccccggcccatttcctacttgaaaggctcctcggggggtccgctgctgtgccccgcgggacacgccgtaggcttattcagggccgcggtgtgcacccgtggagtggctaaggcggtggacttcatccctgtggagaacctagagacaaccatgaggtccccggtgttcacggacaactcctctccaccagcagtgccccagagcttccaggtgggccacctgcatgctcccaccggcagcggcaaaagcaccaaggtcccggctgcatacgcagctcagggctataaggtgctagtgctcaacccctctgtcgctgcaacactgggctttggtgcttacatgtccaaggcccatggggtcgatcctaatatcaggaccggggtgagaacaattaccactggcagccccatcacgtactccacctacggcaagttccttgccgacggcgggtgttcagggggtgcttatgacataataatttgtgacgagtgccactccacggatgccacatccatcttgggcatcggcaccgttcttgaccaagcagagaccgcgggggcgagactggttgtgctcgccaccgctacccctccgggctccatcaccgtgccccatcctaacatcgaggaggttgctctgtccactaccggagagatccctttttacggcaaggctatccccctcgaggcgatcaagggggggagacatctcatcttctgtcactcaaagaagaagtgcgacgagctcgccgcaaagctggtcgcattgggcatcaatgccgtggcctactaccgcggtcttgacgtgtctgtcatcccaaccagcggcgatgttgtcgtcgtggcgaccgatgctcttatgactggctataccggcgactttgactcggtgatagactgcaacacgtgtgtcacccagacagtcgacctcagccttgaccctaccttcaccattgagacgaccacgctcccccaggacgctgtctcccgcacacaacgccggggcaggactggcagggggaagccaggcatctacagattcgtggcactgggggagcgcccctccggcatgttcgactcgtccgttctctgtgagtgctatgacgcgggctgtgcttggtatgagctcacgcccgccgagactacagttagactacgagcgtacatgaacaccccggggctccctgtgtgccaggaccatcttgaattttgggagggcgtctttacaggcctcacccatatagatgcccatttcctatctcagacaaagcagagcggggaaaactttccttacctggtagcataccaagcaaccgtgtgcgctagggctcaagcccctcccccatcgtgggaccagatgtggaagtgtttgactcgcctcaagcccaccctccatgggccaacacccttgctatacagactgggcgctgttcagaatgaagtcaccctgacgcacccaatcaccaaatacatcatgacatgcatgtcggccgacctggaggtcgtcacgagcacctgggtgctcgtcggcggcgtcctggccgctttggcctcgtattgcctgtcaacaggctgcgtggtcatagtgggcaggattgtcctgtctgggaagccggcaattatacctgacagggaagttctctaccgggagttcgatgagatggaagagtgctctcagcacttaccgtacatcgagcaagggatgatgctcgccgagcagttcaagcagaaggccctcggcctcctgcagaccgcgtcccgtcaggcagaggttgtcgcccctgctgtccagaccaactggcaaaaactcgaggccttctgggcgaagcatatgtggaacttcatcagtgggatacactacttggcgggcttgtcaacgttgcctggtaaccccgccattgcttcattgatggcttttacagctgctgtcaccagcccactaaccactagccaaaccctcctcttcaacatactgggggggtgggtggctgcccagcttgccgcccccggtgccgccaccgcctttgtgggcgctggcttagccggcgccgcaatcggcagtgttggactggggaaggtcctcgtggacattctagcagggtatggcgcgggcgtggcgggagctcttgtagcattcaagatcatgagcggtgaggtcccctccacggaggacctagtcaacctgctgcccgccatcctctcgcctggagcccttgtagtcggtgtggtctgcgcagcaatactgcgccggcacgtcggcccgggcgagggggcagtgcaatggatgaaccggctaatcgccttcgcctcccgggggacccatgtttcccccacgcactatgtgccggagagcgatgcagctgcccgcgtcactaccatactcagcagcctcactgtaacccagctcctgaggcgactgcaccagtggataagctcggagtgtaccactccatgctccggttcctggctgagggacatctgggactggatatgcgaggtgctgagcgactttaagacctggctgaaagccaagctcatgccgcaactgcctgggattccctttgtgtcctgccagcgtgggtataagggggtctggcgaggggacggcatcatgcacactcgctgccactgtggagctgagataactggacatgtcaaaaacgggacgatgaggatcgttggtcctaagacttgcaggaacatgtggagtgggactttccccattaacgcctacaccacgggcccctgtactccccttcctgcgccgaactatacgttcgcgctgtggagggtgtctgcagaggaatacgtggagataaggcaggtgggggacttccactacgtgacgggtatgactactgacaaccttaaatgcccgtgccaggtcccatcgcccgaatttttcacagaattggacggggtgcgcctacataggtttgcgcccccttgcaagcccctgctgcgggaggaggtgtcattcagagtgggactccacgagtacccggtggggtcgcaattaccttgcgagcccgaaccggacgtggccgtgttgacgtccatgctcactgatccctcccatataacagcagaggcggccgggagaaggttggcgaggggatcacccccctctatggccagctcctcggctagccaactgtccgctccatctctcagggcaacttgcactaccaaccatgactcccctgatgctgagctcatagaggccaacctcctatggaggcaggagatgggcggcaacatcaccagggttgagtcagagaacaaagtggtgattctggactccttcgatccgcttgtggcagaggaggatgagcgggaggtctccgtgcccgcagagatactgcggaagtctcggaaattcaccccagccctacccatttgggcgcggccggactataaccccccgctggtggagccgtggaaaaagcctgactacgaaccacctgtggtccatggctgcccgcttccacctccacagtcccctcctgtgcctccacctcggaagaagcggacggtgatcctcaccgaatcaaccctacctactgccttggccgagcttgccaccaaaagttttggcagctcctcaacttccggcattacgggcgacgacacgacaacatcccctgagcccgcctcctctagctgccctcccgactccgacgctgagtcctattcttccatgccccctctggagggggagcctggggatccggatctcagcgacgggtcatggtcgacggtcagtagtgaggccgacaaggaggatgtcgtgtgctgctcaatgtcttatacctggacaggcgcactcgtcaccccgtgcgccgcggaagaacaaaaactgcccatcaacgcactaagcaactcgttgctgcgtcatcacaatctggtgtattccaccacctcacgcagtgcttgccaaaggcagaagaaagtcacatttgacagactgcaagtcctggacagccattaccaggacgtgctcaaggaggttaaggcagcggcgtcaaaagtgaaggctaacttgctatccgtagaggaagcttgcagcctgacgcccccacactcagccaaatccaagtttggctatggggcaaaagacgtccgttgccatgccagaaaggccgtaaaccacatcaactccgtgtggaaagaccttctggaagacagtgtaacaccaatagacactaccatcatggctaagaacgaggttttctgcgttcagcctgagaaggggggtcgtaagccagctcgtctcatcgtgttccccgacctgggtgtacgcgtgtgcgagaagatggccttgtacgacgtagtcagcaagctccccctagccgtgatgggaagctcctacggattccaatactcaccaggacagcgggttgaattcctcgtgcaagcgtggaagtccaagaagaccccaatggggttttcgtatgatacccgctgttttgactccacagtcactgagaatgatatccgtacggaggaggcaatctaccaatgttgtgacctggacccccaagcccgcgtggccatcaagtccctcactgagaggctttatgtcgggggccctcttaccaattcaaggggggagaactgcggctatcgcaggtgccgcgcgagcggcgtactgacgaccagctgtggtaacaccctcacctgctacatcaaggcccgagcagcctgtcgagccgcagggctccaggactgcaccatgctcgtgtgtggcgacgacttagtcgttatctgtgagagtgcgggggtccaggaggacgcggcgagcctgagagccttcacggaggctatgaccaggtactccgccccccccggggaccccccacaaccagaatacgacttggagctcataacatcatgctcctccaacgtgtcagtcgcccacgacggcgctggaaaaagggtctactacctcacccgtgaccctacaacccccctcgcgcgggccgcgtgggagacagcaagacacactccagtcaattcctggctaggcaacataattatgtttgcccccacactgtgggcgaggatgatactgatgacccatttctttagcgtcctcatagccagggatcagcttgaacaggccctcgattgcgagatctacggggcctgctactccatagaaccactggatctacctccaatcattcaaagactccatggcctcagcgcattttcactccacagttactctccaggtgaaatcaatagggtggccgcatgcctcagaaaacttggggtcccgcccttgcgagcttggagacaccgggcccggaatgtccgcgctaggcttctgtccagaggaggcagggctgccatttgtggcaagtacctcttcaactgggcagtaaggacaaagctcaaactcactccaatagcggccgctggccggctagacttatctggctggttcacggctggctacagcgggggaggcatttttcacagcgtgtctcatgcccggccccgctggttctggtcttgcctactcctgctcgctgcaggggtaggcatctacctcctccccaaccgatgaaggttggggtaaacactccggcctcttaggccatttcctgttttttttttttttttttttttttttttttttttttttttttttttctttttccctctttttcttctctttttccttctttaatggtggctccatcttagccctagtcacggctagctgtgaaaggtccgtgagccgcatgactgcagagagtgctgatactggcctctctgcagatcatgt

SEQ ID NO: 3 - protein, 3030 aa, Hepatitis C virus
MSTNPKPQRKTKRNTNRRPQDVKFPGGGQIVGGVYLLPRRGPRLGVRATRKTSERSQPRGRRQPIPKARQPTGRSWGQPGYPWPLYANEGLGWAGWLLSPRGSRPNWGPNDPRWKSRNLGKVIDTLTCGFADLMGYIPLVGGPVGGVARALAHGVRVLEDGVNYATGNLPGCSFSIFILALLSCLTAPTSAVPYRNASGVYHVTNDCPNSSIVYEAEDLILHAPGCVPCVRQGNLSRCWVQITPTLSAPSLGAVTAPLRRAVDYLAGGAALCSALYVGDACGAVFLVGQMFTYSPRRHNVVQDCNCSIYSGHITGHRMAWDMMMNWSPTTALVMAQLLRIPQVVIDIIAGAHWGVLFAAAYYASAANWAKVVLVLFLFAGVDASPRTVGGSAAQGARGLASLFTPGPQQNLQLINTNGSWHINRTALNCNDSLQTGFVAGLLYYHKFNSTGCPQRMASCRPLAAFDQGWGTISYAAVSGPSDDKPYCWHYPPRPCGIVPARGVCGPVYCFTPSPVVVGTTDRKGNPTYSWGENETDIFLLNNTRPPTGNWFGCTWMNSTGFVKTCGAPPCNLGPTGNNSLKCPTDCFRKHPDATYTKCGSGPWLTPRCLVHYPYRLWHYPCTLNYTIFKVRMYIGGLEHRLEVACNWTRGERCDLEDRDRAELSPLLHTTTQWAILPCSFTPTPALSTGLIHLHQNIVDTQYLYGLSSSIVSWAVKWEYIVLAFLLLADARICTCLWIMLLVCQAEAALENVIVLNAAAAAGTHGFFWGLLVICFAWHFKGRVVPGATYLCLGIWPLLLLLFLLPQRALALDSSDGGTVGCLVLTILTIFTLTPGYKKMVVLVIWWLQYFIARVEAFIHVWVPPLQVRGGRDAIIMLTCLFHPALGFEVTKILLGILGPLCLLQYSLIKLPYFIRARALLRACLLAKHLACGRYVQAALLHLGRLTGTYIYDHLAPMKDWAASGLRDLAVATEPIIFSPMETKVITWGADTAACGDILAGLPVSARRGHEIFLGPADDIREGGWRLLAPITAYAQQTRGLLGAIVVSMTGRDRTEQAGEVQILSTVSQSFLGTTISGVLWTVYHGAGNKTLAGLRGPVTQMYSSAEGDLVGWPSPPGTRSLEPCKCGAVDLYLVTRNADVIPARRRGDKRGALLSPRPISTLKGSSGGPVLCPRGHVVGLFRAAVCSRGVAKSIDFIPVETLDVVTRSPTFSDNSTPPAVPQTYQVGYLHAPTGSGKSTKVPVAYAAQGYKVLVLNPSVAATLGFGAYLSKAHGINPNIRTGVRTVMTGEAITYSTYGKFLADGGCASGAYDIIICDECHAVDATSILGIGTVLDQAETAGVRLTVLATATPPGSVTTPHPDIEEVGLGREGEIPFYGRAIPLSCIKGGRHLIFCHSKKKCDELAAALRGMGLNAVAYYRGLDVSIIPAQGDVVVVATDALMTGYTGDFDSVIDCNVAVTQAVDFSLDPTFTITTQTVPQDAVSRSQRRGRTGRGRQGTYRYVSTGERASGMFDSVVLCECYDAGAAWYDLTPAETTVRLRAYFNTPGLPVCQDHLEFWEAVFTGLTHIDAHFLSQTKQAGENFAYLVAYQATVCARAKAPPPSWDAMWKCLARLKPTLAGPTPLLYRLGPITNEVTLTHPGTKYIATCMQADLEVMTSTWVLAGGVLAAVAAYCLATGCVSIIGRLHVNQRVVVAPDKEVLYEAFDEMEECASRAALIEEGQRIAEMLKSKIQGLLQQASKQAQDIQPAMQASWPKVEQFWARHMWNFISGIQYLAGLSTLPGNPAVASMMAFSAALTSPLSTSTTILLNIMGGWLASQIAPPAGATGFVVSGLVGAAVGSIGLGKVLVDILAGYGAGISGALVAFKIMSGEKPSMEDVINLLPGILSPGALVVGVICAAILRRHVGPGEGAVQWMNRLIAFASRGNHVAPTHYVTESDASQRVTQLLGSLTITSLLRRLHNWITEDCPIPCSGSWLRDVWDWVCTILTDFKNWLTSKLFPKLPGLPFISCQKGYKGVWAGTGIMTTRCPCGADISGNVRLGSMRITGPKTCMNTWQGTFPINCYTEGQCAPKPPTNYKTAIWRVAASEYAEVTQHGSYSYVTGLTTDNLKIPCQLPSPEFFSWVDGVQIHRFAPTPKPFFRDEVSFCVGLNSYAVGSQLPCEPEPDADVLRSMLTDPPHITAETAARRLARGSPPSEASSSVSQLSAPSLRATCTTHSNTYDVDMVDANLLMGGGVAQTEPESRVPALDFLEPMAEEESDPEPSIPSECMLPRSGFPRALPAWARPDYNPPLVESWRRPDYQPPTVAGCALPPPKKAPTPPPRRRRTVGLSESTTSEALQQLAIKTFGQPPSSGDAGSSTGAGAAESGGPTSPGEPAPSETGSASSMPPLEGEPGDPDLESDQVELQPPPQGGGVAPGSGSGSWSTCSEEDDTTVCCSMSYSWTGALITPCSPEEEKLPINPLSNSLLRYHNKVYCTTSKSASQRAKKVTFDRTQVLDAHYDSVLKDIKLAASKVSSRLLTLEEACQLTPPHSARSKYGFGAKEVRSLSGRAVNHIKSVWKDLLEDPQTPIPTTIMAKNEVFCVDPAKGGKKPARLIVYPDLGVRVCEKMALYDITQKLPQAVMGASYGFQYSPAQRVEYLLKAWAEKKDPMGFSYDTRCFDSTVTERDIRTEESIYQACSLPEEARTAIHSLTERLYVGGPMFNSKGQTCGYRRCRASGVLTTSMGNTITCYVKALAACKAAGIVAPTMLVCGDDLVVISESQGTEEDERNLRAFTEAMTRYSAPPGDPPRPEYDLELITSCSSNVSVALGPRGRRRYYLTRDPTTPLARAAWETVRHSPINSWLGNIIQYAPTIWARMVLMTHFFSILMVQDTLDQNLNFEMYGSVYSVNPLDLPAIIERLHGLDAFSMHTYSHHELTRVASALRKLGAPPLRVWKSRARAVRASLISRGGKAAVCGRYLFNWAVKTKLKLTPLPEARLLDLSSWFTVGAGGGDIFHSVSRARPRSLLFGLLLLFVGVGLFLLPAR

SEQ ID NO: 4 - DNA, 9669 bp, Hepatitis C virus
acctgcccctaataggggcgacactccgccatgaatcactcccctgtgaggaactactgtcttcacgcagaaagcgcctagccatggcgttagtatgagtgtcgtacagcctccaggcccccccctcccgggagagccatagtggtctgcggaaccggtgagtacaccggaattgccgggaagactgggtcctttcttggataaacccactctatgcccggccatttgggcgtgcccccgcaagactgctagccgagtagcgttgggttgcgaaaggccttgtggtactgcctgatagggcgcttgcgagtgccccgggaggtctcgtagaccgtgcaccatgagcacgaatcctaaacctcaaagaaaaaccaaaagaaacaccaaccgccgcccacaggacgtcaagttcccgggcggtggtcagatcgttggtggagtttacttgttgccgcgcaggggccctaggttgggtgtgcgcgcaactcggaagacttcagaacggtcgcaaccccgtggacggcgtcagcctatccccaaggcgcgccagcccacgggccggtcctggggtcaacccgggtacccttggcccctttatgccaatgagggcctcgggtgggcagggtggttgctctccccccgaggctctcggcctaattggggccccaatgacccccggtggaaatcgcgcaacttgggtaaggtcatcgataccctgacgtgcggattcgccgacctcatggggtacatcccgctcgtaggcggccccgttgggggcgtcgcaagggctctcgcacacggtgtgagggtccttgaggacggggtaaactatgcaacagggaatttacccggttgctctttctctatctttatccttgcacttctttcatgcctgactgccccgacctctgccgttccctaccgaaatgcctctggggtttatcatgtcaccaatgattgcccaaactcttctatcgtctatgaggctgaagacctgatcttacacgcacctggttgcgtgccctgtgttaggcagggtaatctcagtaggtgctgggtccagatcacccccacactgtcagccccgagcctcggagcggtcacggctcctcttcggagggccgttgactacttagcggggggggctgccctttgctccgcgttatacgtcggagacgcgtgcggggcagtgtttttggtaggtcaaatgttcacctatagccctcgccggcataatgttgtgcaggactgcaactgttccatttacagtggccacatcaccggccaccggatggcatgggacatgatgatgaattggtcacctacaacagctttggtgatggcccagttgttacggattccccaggtggtcattgacatcattgccggggcccactggggggtcttgttcgccgccgcatactacgcgtcggcggctaactgggccaaggttgtgctggtcctgtttctgtttgcgggggtcgatgccagcccccgcactgtgggtggtagtgcggcccaaggcgcgcgcgggctcgcttcacttttcacccctgggccgcagcagaacttgcagctcataaataccaacgggagctggcacatcaacagaactgcccttaactgtaatgacagcctccagactgggtttgtagccggcctcctgtattatcacaagttcaactccactgggtgtccgcagcggatggctagctgtaggcccctcgccgcattcgaccagggctggggaactatcagctatgccgccgtgtcgggccccagtgatgacaagccctattgctggcactaccccccacgcccgtgcggaatagtgccagcgcgaggtgtctgcggtccggtctattgttttacacctagcccggtggtcgtcggcaccacagaccgcaaggggaatcccacttacagttggggcgaaaatgagactgacatctttctcttgaacaacacgaggccccctactggcaactggtttggctgcacctggatgaattccacagggtttgtcaagacttgcggggctccaccctgcaacttagggcctacaggcaacaatagccttaagtgtcctactgattgcttccgcaagcacccagacgccacctacaccaagtgtgggtcaggaccctggctcactccccggtgtctggtgcattacccttaccggttgtggcattacccgtgcaccctaaattacaccatcttcaaggtgcgcatgtacattgggggcctcgagcacaggctcgaggtggcatgcaactggacccgtggtgagcggtgtgatcttgaagacagggatagggccgagctgagcccgctcctacataccaccacgcagtgggccatattgccgtgctctttcacacccacacccgctcttagcactggtctcatacacttacatcaaaatatagtagacacccagtatctttacggtctgagctccagcatcgtctcgtgggccgttaagtgggagtacatagtgctggccttcttattacttgctgatgcccgtatttgtacttgcctatggatcatgctcctggtttgtcaggccgaagcggccctggagaacgtcattgtcctaaacgcggctgcggctgcggggactcatgggtttttctggggcctgctcgtcatctgcttcgcctggcacttcaagggcagggtggtccctggggccacctacctttgcttgggcatttggccattactcttactccttttcctcctgccccaaagggctctagccctggactcaagcgatggcgggactgtgggttgtcttgtgttaaccatccttacaatcttcacactcacccccgggtacaagaagatggtagtgttggtcatatggtggcttcagtatttcatagcccgggtagaggcctttatccatgtgtgggtgcccccgttgcaggttaggggtggtcgtgatgctattatcatgctcacatgccttttccatcctgccctggggtttgaggtcacgaaaatcctcctcgggatactaggtcctttgtgcctgctgcagtactcgctcatcaagctgccttatttcatcagggcgcgcgccctgctgagggcgtgcctgctagcgaagcacttggcctgtggcaggtacgtgcaggcggccttgctccaccttggtaggctgaccggaacgtacatttatgaccaccttgcccccatgaaggattgggcagcgtccgggctgcgcgacttagcagtggccacggagcccatcatattctcccctatggagacgaaggtcatcacgtggggggctgacacggccgcatgtggggacatacttgccggccttcctgtatcagctaggcgaggccatgaaatcttcctggggccagccgatgacatcagagaggggggctggcgacttctcgctcccatcactgcttatgcccagcaaacacgaggcctcctgggcgccatagtggtgagtatgacggggcgtgacaggacagaacaggccggggaagtccaaatcctgtccacagtctctcagtccttcctcggaacaaccatctcgggggttttgtggactgtttaccacggagctggcaacaagactctagccggcttacggggtccggtcacgcagatgtactcgagtgctgagggggacttggtaggctggcccagcccccctgggaccaggtctttggagccgtgcaagtgtggagccgtcgacctatatctggtcacgcggaacgctgatgtcatcccggctcggagacgcggggacaagcggggagcattgctctccccgagacccatttcgaccttgaaggggtcctcgggggggccggtgctctgccctaggggccacgtcgttgggctcttccgagcagctgtgtgctctcggggcgtggccaaatccatcgatttcatccccgttgagacactcgacgttgttacaaggtctcccactttcagtgacaacagcacgccaccggctgtgccccagacctatcaggtcgggtacttgcatgctccaactggcagtggaaagagcaccaaggtccctgtcgcgtatgccgcccaggggtacaaagtactagtgcttaacccctcggtagctgccaccctggggtttggggcgtacctatccaaggcacatggcatcaatcccaacattaggactggagtcaggaccgtgatgaccggggaggccatcacgtactccacatatggcaaatttctcgccgatgggggctgcgctagcggcgcctatgacatcatcatatgcgatgaatgccacgctgtggatgctacctccattctcggcatcggaacggtccttgatcaagcagagacagccggggtcagactaactgtgctggctacggccacaccccccgggtcagtgacaaccccccatcccgatatagaagaggtaggcctcgggcgggagggtgagatccccttctatgggagggcgattcccctatcctgcatcaagggagggagacacctgattttctgccactcaaagaaaaagtgtgacgagctcgcggcggcccttcggggcatgggcttgaatgccgtggcatactatagagggttggacgtctccataataccagctcagggagatgtggtggtcgtcgccaccgacgccctcatgacggggtacactggagactttgactccgtgatcgactgcaatgtagcggtcacccaagctgtcgacttcagcctggaccccaccttcactataaccacacagactgtcccacaagacgctgtctcacgcagtcagcgccgcgggcgcacaggtagaggaagacagggcacttataggtatgtttccactggtgaacgagcctcaggaatgtttgacagtgtagtgctttgtgagtgctacgacgcaggggctgcgtggtacgatctcacaccagcggagaccaccgtcaggcttagagcgtatttcaacacgcccggcctacccgtgtgtcaagaccatcttgaattttgggaggcagttttcaccggcctcacacacatagacgcccacttcctctcccaaacaaagcaagcgggggagaacttcgcgtacctagtagcctaccaagctacggtgtgcgccagagccaaggcccctcccccgtcctgggacgccatgtggaagtgcctggcccgactcaagcctacgcttgcgggccccacacctctcctgtaccgtttgggccctattaccaatgaggtcaccctcacacaccctgggacgaagtacatcgccacatgcatgcaagctgaccttgaggtcatgaccagcacgtgggtcctagctggaggagtcctggcagccgtcgccgcatattgcctggcgactggatgcgtttccatcatcggccgcttgcacgtcaaccagcgagtcgtcgttgcgccggataaggaggtcctgtatgaggcttttgatgagatggaggaatgcgcctctagggcggctctcatcgaagaggggcagcggatagccgagatgttgaagtccaagatccaaggcttgctgcagcaggcctctaagcaggcccaggacatacaacccgctatgcaggcttcatggcccaaagtggaacaattttgggccagacacatgtggaacttcattagcggcatccaatacctcgcaggattgtcaacactgccagggaaccccgcggtggcttccatgatggcattcagtgccgccctcaccagtccgttgtcgaccagtaccaccatccttctcaacatcatgggaggctggttagcgtcccagatcgcaccacccgcgggggccaccggctttgtcgtcagtggcctggtgggggctgccgtgggcagcataggcctgggtaaggtgctggtggacatcctggcaggatatggtgcgggcatttcgggggccctcgtcgcattcaagatcatgtctggcgagaagccctctatggaagatgtcatcaatctactgcctgggatcctgtctccgggagccctggtggtgggggtcatctgcgcggccattctgcgccgccacgtgggaccgggggagggcgcggtccaatggatgaacaggcttattgcctttgcttccagaggaaaccacgtcgcccctactcactacgtgacggagtcggatgcgtcgcagcgtgtgacccaactacttggctctcttactataaccagcctactcagaagactccacaattggataactgaggactgccccatcccatgctccggatcctggctccgcgacgtgtgggactgggtttgcaccatcttgacagacttcaaaaattggctgacctctaaattgttccccaagctgcccggcctccccttcatctcttgtcaaaaggggtacaagggtgtgtgggccggcactggcatcatgaccacgcgctgcccttgcggcgccgacatctctggcaatgtccgcctgggctctatgaggatcacagggcctaaaacctgcatgaacacctggcaggggacctttcctatcaattgctacacggagggccagtgcgcgccgaaaccccccacgaactacaagaccgccatctggagggtggcggcctcggagtacgcggaggtgacgcagcatgggtcgtactcctatgtaacaggactgaccactgacaatctgaaaattccttgccaactaccttctccagagtttttctcctgggtggacggtgtgcagatccataggtttgcacccacaccaaagccgtttttccgggatgaggtctcgttctgcgttgggcttaattcctatgctgtcgggtcccagcttccctgtgaacctgagcccgacgcagacgtattgaggtccatgctaacagatccgccccacatcacggcggagactgcggcgcggcgcttggcacggggatcacctccatctgaggcgagctcctcagtgagccagctatcagcaccgtcgctgcgggccacctgcaccacccacagcaacacctatgacgtggacatggtcgatgccaacctgctcatggggggcggtgtggctcagacagagcctgagtccagggtgcccgctctggactttctcgagccaatggccgaggaagagagcgaccctgagccctcaataccatcggagtgcatgctccccaggagcgggtttccacgggccttaccggcttgggcacggcctgactacaacccgccgctcgtggaatcgtggaggaggccagattaccaaccgcccaccgttgctggttgtgctctccccccccccaagaaggccccgacgcctcccccaaggagacgccggacagtgggtctgagcgagagcaccacatcagaagccctccagcaactggccatcaagacctttggccagcccccctcgagcggtgatgcaggctcgtccacgggggcgggcgccgccgaatccggcggtccgacgtcccctggtgagccggccccctcagagacaggttccgcctcctctatgccccccctcgagggggagcctggagatccggacctggagtctgatcaggtagagcttcaacctcccccccagggggggggggtagctcccggttcgggctcggggtcttggtctacttgctccgaggaggacgataccaccgtgtgctgctccatgtcatactcctggaccggggctctaataactccctgtagccccgaagaggaaaagttgccaatcaaccctttgagtaactcgctgttgcgataccataacaaggtgtactgtacaacatcaaagagcgcctcacagagggctaaaaaggtaacttttgacaggacgcaagtgctcgacgcccattatgactcagtcttaaaggacatcaagctagcggcttccaaggtcagctcgaggctcctcaccttggaggaggcgtgccagttgactccaccccattctgcaagatccaagtatggattcggggccaaggaggtccgcagcttgtccgggagggccgttaaccacatcaagtccgtgtggaaggacctcctggaagacccacaaacaccaattcccacaaccatcatggccaaaaatgaggtgttctgcgtggaccccgccaaggggggtaagaaaccagctcgcctcatcgtttaccctgacctcggcgtccgggtctgcgagaaaatggccctctatgacattacacaaaagcttcctcaggcggtaatgggagcttcctatggcttccagtactcccctgcccaacgggtggagtatctcttgaaagcatgggcggaaaagaaggaccccatgggtttttcgtatgatacccgatgcttcgactcaaccgtcactgagagagacatcaggaccgaggagtccatataccaggcctgctccctgcccgaggaggcccgcactgccatacactcgctgactgagagactttacgtaggagggcccatgttcaacagcaagggtcaaacctgcggttacagacgttgccgcgccagcggggtgctaaccactagcatgggtaacaccatcacatgctatgtgaaagccctagcggcctgcaaggctgcggggatagttgcgcccacaatgctggtatgcggcgatgacctagtagtcatctcagaaagccaggggactgaggaggacgagcggaacctgagagccttcacggaggccatgaccaggtactctgcccctcctggtgatccccccagaccggaatatgacctggagctaataacatcctgttcctcaaatgtgtctgtggcgttgggcccgcggggccgccgcagatactacctgaccagagacccaaccactccactcgcccgggctgcctgggaaacagttagacactcccctatcaattcatggctgggaaacatcatccagtatgctccaaccatatgggctcgcatggtcctaatgacacacttcttctccattctcatggtccaagacaccctggaccagaacctcaactttgagatgtatggatcagtatactccgtgaatcctttggaccttccagccataattgagaggttacacgggcttgacgccttttctatgcacacatactctcaccacgaactgacgcgggtggcttcagccctcagaaaacttggggcgccacccctcagggtgtggaagagtcgggctcgcgcagtcagggcgtccctcatctcccgtggagggaaagcggccgtttgcggccgatatctcttcaattgggcggtgaagaccaagctcaaactcactccattgccggaggcgcgcctactggacttatccagttggttcaccgtcggcgccggcgggggcgacatttttcacagcgtgtcgcgcgcccgaccccgctcattactcttcggcctactcctacttttcgtaggggtaggcctcttcctactccccgctcggtagagcggcacacactaggtacactccatagctaactgttcctttttttttttttttttttttttttttttttttttttttttttcttttttttttttttccctctttcttcccttctcatcttattctactttctttcttggtggctccatcttagccctagtcacggctagctgtgaaaggtccgtgagccgcatgactgcagagagtgccgtaactggtctctctgcagatcatgt

SEQ ID NO: 5 - DNA, 18 bp, Artificial Sequence
  Probe used for HCV quantification
ccttgtggtactgcctga

SEQ ID NO: 6 - DNA, 18 bp, Artificial Sequence
  Forward primer used for HCV quantification
agygttgggtygcgaaag

SEQ ID NO: 7 - DNA, 16 bp, Artificial Sequence
  Reverse primer used for HCV quantification
cactcgcaagcrccct